European Patent Application EP 4 417 690 A1, published August 21, 2024. Title: 转氨酶突变体及手性胺化合物的制备方法. Applicant: 凯莱英生命科学技术（天津）有限公司. The sequence listing filed with the application follows.

SEQUENCE LISTING (3 sequences)

SEQ ID NO: 1 - protein, 459 aa, synthetic construct
  source 1..459: note; note (original language) = 来源于Chromobaterium violaceum的氨基酸突变体
MQKQRTCSQWRELDAAHHLHPFTDTASLNQAGARVMTRGEGVYLWDCEGNKIIDGMAGAWCVNVGYGRKDFAEAARRQMEELPFYNTAYKTTHPAVVELSSLLAEVTPAGFDRVFYTNSGSESVDTMIRMVRRYWDVQGKPEKKTLIGRWNGYHGSTIGGASLGGFKEMHEQGDLPIPGMAHIEQPWWYKHGKDMTPDEFGVVAARWLEEKILEIGADKVAAFVGEPIQGAGGVIVPPATYWPEIERICRKYDVLLVADEVICGFGRTGEWFGHQHFGFQPDLFTAAKGLSSGYLPIGAVFVGKRVAEGLIAGGDFNHGFTYSGHPVCAAVAHANVAALRDEGIVQRVKDDIGPYMQKRWRETFSRFEHVDDVRGVGMLLAFTLVKNKAKRELFPDFGEIGTLCRDIFFRNNLIMDSCGDHIVSAPPLVMTRAEVDEMLAVAERCLEEFEQTLKARGLA

SEQ ID NO: 2 - protein, 459 aa, synthetic construct
  source 1..459: note = V234A
MQKQRTCSQWRELDAAHHLHPFTDTASLNQAGARVMTRGEGVYLWDCEGNKIIDGMAGAWCVNVGYGRKDFAEAARRQMEELPFYNTAYKTTHPAVVELSSLLAEVTPAGFDRVFYTNSGSESVDTMIRMVRRYWDVQGKPEKKTLIGRWNGYHGSTIGGASLGGFKEMHEQGDLPIPGMAHIEQPWWYKHGKDMTPDEFGVVAARWLEEKILEIGADKVAAFVGEPIQGAGGAIVPPATYWPEIERICRKYDVLLVADEVICGFGRTGEWFGHQHFGFQPDLFTAAKGLSSGYLPIGAVFVGKRVAEGLIAGGDFNHGFTYSGHPVCAAVAHANVAALRDEGIVQRVKDDIGPYMQKRWRETFSRFEHVDDVRGVGMLLAFTLVKNKAKRELFPDFGEIGTLCRDIFFRNNLIMDSCGDHIVSAPPLVMTRAEVDEMLAVAERCLEEFEQTLKARGLA

SEQ ID NO: 3 - protein, 459 aa, synthetic construct
  source 1..459: note = V234C
MQKQRTCSQWRELDAAHHLHPFTDTASLNQAGARVMTRGEGVYLWDCEGNKIIDGMAGAWCVNVGYGRKDFAEAARRQMEELPFYNTAYKTTHPAVVELSSLLAEVTPAGFDRVFYTNSGSESVDTMIRMVRRYWDVQGKPEKKTLIGRWNGYHGSTIGGASLGGFKEMHEQGDLPIPGMAHIEQPWWYKHGKDMTPDEFGVVAARWLEEKILEIGADKVAAFVGEPIQGAGGCIVPPATYWPEIERICRKYDVLLVADEVICGFGRTGEWFGHQHFGFQPDLFTAAKGLSSGYLPIGAVFVGKRVAEGLIAGGDFNHGFTYSGHPVCAAVAHANVAALRDEGIVQRVKDDIGPYMQKRWRETFSRFEHVDDVRGVGMLLAFTLVKNKAKRELFPDFGEIGTLCRDIFFRNNLIMDSCGDHIVSAPPLVMTRAEVDEMLAVAERCLEEFEQTLKARGLA